European Patent Application EP 4 548 937 A1, published May 7, 2025. Title: Antibody-Drug Conjugate. Applicant: Eisai R&D Management Co., Ltd. The sequence listing filed with the application follows.

SEQUENCE LISTING (61 sequences)

SEQ ID NO: 1 - protein, 344 aa, Human CEACAM6
MGPPSAPPCRLHVPWKEVLLTASLLTFWNPPTTAKLTIESTPFNVAEGKEVLLLAHNLPQNRIGYSWYKGERVDGNSLIVGYVIGTQQATPGPAYSGRETIYPNASLLIQNVTQNDTGFYTLQVIKSDLVNEEATGQFHVYPELPKPSISSNNSNPVEDKDAVAFTCEPEVQNTTYLWWVNGQSLPVSPRLQLSNGNMTLTLLSVKRNDAGSYECEIQNPASANRSDPVTLNVLYGPDVPTISPSKANYRPGENLNLSCHAASNPPAQYSWFINGTFQQSTQELFIPNITVNNSGSYMCQAHNSATGLNRTTVTMITVSGSAPVLSAVATVGITIGVLARVALI

SEQ ID NO: 2 - protein, 286 aa, Human CEACAM6 extracellular region
KLTIESTPFNVAEGKEVLLLAHNLPQNRIGYSWYKGERVDGNSLIVGYVIGTQQATPGPAYSGRETIYPNASLLIQNVTQNDTGFYTLQVIKSDLVNEEATGQFHVYPELPKPSISSNNSNPVEDKDAVAFTCEPEVQNTTYLWWVNGQSLPVSPRLQLSNGNMTLTLLSVKRNDAGSYECEIQNPASANRSDPVTLNVLYGPDGPTISPSKANYRPGENLNLSCHAASNPPAQYSWFINGTFQQSTQELFIPNITVNNSGSYMCQAHNSATGLNRTTVTMITVSG

SEQ ID NO: 3 - protein, 788 aa, Human CEACAM6 extracellular domain - SEAP-His protein
KLTIESTPFNVAEGKEVLLLAHNLPQNRIGYSWYKGERVDGNSLIVGYVIGTQQATPGPAYSGRETIYPNASLLIQNVTQNDTGFYTLQVIKSDLVNEEATGQFHVYPELPKPSISSNNSNPVEDKDAVAFTCEPEVQNTTYLWWVNGQSLPVSPRLQLSNGNMTLTLLSVKRNDAGSYECEIQNPASANRSDPVTLNVLYGPDGPTISPSKANYRPGENLNLSCHAASNPPAQYSWFINGTFQQSTQELFIPNITVNNSGSYMCQAHNSATGLNRTTVTMITVSGAAAIIPVEEENPDFWNREAAEALGAAKKLQPAQTAAKNLIIFLGDGMGVSTVTAARILKGQKKDKLGPEIPLAMDRFPYVALSKTYNVDKHVPDSGATATAYLCGVKGNFQTIGLSAAARFNQCNTTRGNEVISVMNRAKKAGKSVGVVTTTRVQHASPAGTYAHTVNRNWYSDADVPASARQEGCQDIATQLISNMDIDVILGGGRKYMFRMGTPDPEYPDDYSQGGTRLDGKNLVQEWLAKRQGARYVWNRTELMQASLDPSVTHLMGLFEPGDMKYEIHRDSTLDPSLMEMTEAALRLLSRNPRGFFLFVEGGRIDHGHHESRAYRALTETIMFDDAIERAGQLTSEEDTLSLVTADHSHVFSFGGYPLRGSSIFGLAPGKARDRKAYTVLLYGNGPGYVLKDGARPDVTESESGSPEYRQQSAVPLDEETHAGEDVAVFARGPQAHLVHGVQEQTFIAHVMAFAACLEPYTACDLAPPAGTTDAAHPGHHHHHHHHHH

SEQ ID NO: 4 - protein, 663 aa, Human CEACAM6 extracellular domain - MBP-His protein
KLTIESTPFNVAEGKEVLLLAHNLPQNRIGYSWYKGERVDGNSLIVGYVIGTQQATPGPAYSGRETIYPNASLLIQNVTQNDTGFYTLQVIKSDLVNEEATGQFHVYPELPKPSISSNNSNPVEDKDAVAFTCEPEVQNTTYLWWVNGQSLPVSPRLQLSNGNMTLTLLSVKRNDAGSYECEIQNPASANRSDPVTLNVLYGPDGPTISPSKANYRPGENLNLSCHAASNPPAQYSWFINGTFQQSTQELFIPNITVNNSGSYMCQAHNSATGLNRTTVTMITVSGAAAEEGKLVIWINGDKGYNGLAEVGKKFEKDTGIKVTVEHPDKLEEKFPQVAATGDGPDIIFWAHDRFGGYAQSGLLAEITPDKAFQDKLYPFTWDAVRYNGKLIAYPIAVEALSLIYNKDLLPNPPKTWEEIPALDKELKAKGKSALMFNLQEPYFTWPLIAADGGYAFKYENGKYDIKDVGVDNAGAKAGLTFLVDLIKNKHMNADTDYSIAEAAFNKGETAMTINGPWAWSNIDTSKVNYGVTVLPTFKGQPSKPFVGVLSAGINAASPNKELAKEFLENYLLTDEGLEAVNKDKPLGAVALKSYEEELAKDPRIAATMENAQKGEIMPNIPQMSAFWYAVRTAVINAASGRQTVDEALKDAQTHHHHHHHHHH

SEQ ID NO: 5 - protein, 19 aa, synthetic construct
  REGION 1..19: note = Signal sequence
MEWSWVFLFFLSVTTGVHS

SEQ ID NO: 6 - protein, 120 aa, synthetic construct
  REGION 1..120: note = Antibody A heavy chain variable region amino acid sequence
EVQLLESGGGLVQPGGSLRLSCAASGFTFSSYAMSWVRQAPGKGLEWVSAISGSGGSTYYADSVKGRFTISRDNSKNTLYLQMNSLRAEDTAVYYCARYWIWWHYGFDVWGQGTLVTVSS

SEQ ID NO: 7 - protein, 108 aa, synthetic construct
  REGION 1..108: note = Antibody A light chain variable region amino acid sequence
SSELTQDPAVSVALGQTVRITCQGDSLRSYYASWYQQKPGQAPVLVIYGKNNRPSGIPDRFSGSSSGNTASLTITGAQAEDEADYYCQSYYSSSHYVVFGGGTKLTVL

SEQ ID NO: 8 - DNA, 360 bp, synthetic construct
  misc_feature 1..360: note = Antibody A heavy chain variable region gene acid sequence
  source 1..360: mol_type = other DNA
gaagtgcagctgctggaatccgggggagggctggtgcagcccggcggctctctgagactgtcctgtgctgcctccggcttcaccttttccagctacgctatgtcttgggtgcggcaggctcctggcaagggactggagtgggtgtctgctatcagcggctctggcggctccacatactatgccgacagcgtgaagggcaggttcaccatctctcgggataactccaagaatacactgtatctgcagatgaactctctgagggctgaggacaccgccgtgtactattgcgctcggtactggatctggtggcactatggatttgacgtgtggggacagggcaccctggtgacagtgtcttcc

SEQ ID NO: 9 - DNA, 324 bp, synthetic construct
  misc_feature 1..324: note = Antibody A light chain variable region gene acid sequence
  source 1..324: mol_type = other DNA
tctagtgaactgacccaggatcccgccgtctctgtggccctgggccagacagtgagaatcacctgccagggcgactctctgcgctcctactatgcctcttggtaccagcagaagccaggccaggctcccgtgctggtcatctacggcaagaacaataggccttccggcatcccagatcggtttagcggctccagctctggcaacacagccagcctgacaattacaggagctcaggctgaggatgaggctgattactattgccagtcttactattccagctctcactacgtggtgttcgggggagggacaaagctgaccgtgctg

SEQ ID NO: 10 - protein, 329 aa, Human IgG1/2m amino acid sequence
ASTKGPSVFPLAPSSKSTSGGTAALGCLVKDYFPEPVTVSWNSGALTSGVHTFPAVLQSSGLYSLSSVVTVPSSSLGTQTYICNVNHKPSNTKVDKRVEPKSCDKTHTCPPCPAPPAAAPSVFLFPPKPKDTLMISRTPEVTCVVVDVSHEDPEVQFNWYVDGVEVHNAKTKPREEQFNSTFRVVSVLTVVHQDWLNGKEYKCKVSNKGLPAPIEKTISKTKGQPREPQVYTLPPSREEMTKNQVSLTCLVKGFYPSDIAVEWESNGQPENNYKTTPPMLDSDGSFFLYSKLTVDKSRWQQGNVFSCSVMHEALHNHYTQKSLSLSPGK

SEQ ID NO: 11 - protein, 106 aa, Human Ig amino acid sequence
GQPKAAPSVTLFPPSSEELQANKATLVCLISDFYPGAVTVAWKADSSPVKAGVETTTPSKQSNNKYAASSYLSLTPEQWKSHRSYSCQVTHEGSTVEKTVAPTECS

SEQ ID NO: 12 - DNA, 987 bp, Human IgG1/2m gene acid sequence
  source 1..987: mol_type = genomic DNA
gcctccacaaagggaccatccgtgttcccactggccccaagctctaagtccaccagcggcggcacagccgctctgggctgtctggtgaaggactacttccctgagccagtgaccgtgagctggaactctggcgctctgacctccggcgtgcatacatttccagccgtgctgcagtccagcggcctgtacagcctgtcttccgtggtgaccgtgcccagctcttccctgggcacccagacatatatctgcaacgtgaatcacaagcctagcaatacaaaggtggacaagagagtggagccaaagtcttgtgataagacccatacatgccctccatgtcctgccccacccgccgctgccccttccgtgttcctgtttcctccaaagccaaaggacaccctgatgatctctcgcacccctgaggtgacatgcgtggtggtggacgtgagccacgaggatcctgaggtgcagtttaactggtacgtggatggcgtggaggtgcataatgctaagacaaagccaagagaggagcagttcaactctacctttcgcgtggtgtccgtgctgacagtggtgcaccaggattggctgaacggcaaggagtataagtgcaaggtgtctaataagggcctgcccgcccctatcgagaagaccatctccaagacaaagggccagcctagagagccacaggtgtacaccctgcccccttctcgcgaggagatgaccaagaaccaggtgtccctgacatgtctggtgaagggcttctatccctccgacatcgctgtggagtgggagagcaatggccagcctgagaacaattacaagaccacaccacccatgctggactccgatggcagcttctttctgtatagcaagctgaccgtggataagtctaggtggcagcagggcaacgtgttctcctgttccgtgatgcacgaagccctgcacaaccattatactcagaagagcctgtccctgtcccctggcaaa

SEQ ID NO: 13 - DNA, 318 bp, Human Ig gene acid sequence
  source 1..318: mol_type = genomic DNA
ggacagccaaaggctgctccttctgtgaccctgtttcccccttccagcgaggagctgcaggccaataaggccaccctggtgtgcctgatcagcgacttctatccaggagctgtgacagtggcttggaaggctgattcttccccagtgaaggctggcgtggagaccacaacccccagcaagcagtctaacaataagtacgccgcctcctcttatctgtctctgacaccagagcagtggaagtcccataggtcctacagctgccaggtgacccacgaaggtagcacagtcgaaaaaaccgtcgcccccacagagtgttct

SEQ ID NO: 14 - protein, 449 aa, synthetic construct
  REGION 1..449: note = Antibody A heavy chain full-length amino acid sequence (no signalsequence)
EVQLLESGGGLVQPGGSLRLSCAASGFTFSSYAMSWVRQAPGKGLEWVSAISGSGGSTYYADSVKGRFTISRDNSKNTLYLQMNSLRAEDTAVYYCARYWIWWHYGFDVWGQGTLVTVSSASTKGPSVFPLAPSSKSTSGGTAALGCLVKDYFPEPVTVSWNSGALTSGVHTFPAVLQSSGLYSLSSVVTVPSSSLGTQTYICNVNHKPSNTKVDKRVEPKSCDKTHTCPPCPAPPAAAPSVFLFPPKPKDTLMISRTPEVTCVVVDVSHEDPEVQFNWYVDGVEVHNAKTKPREEQFNSTFRVVSVLTVVHQDWLNGKEYKCKVSNKGLPAPIEKTISKTKGQPREPQVYTLPPSREEMTKNQVSLTCLVKGFYPSDIAVEWESNGQPENNYKTTPPMLDSDGSFFLYSKLTVDKSRWQQGNVFSCSVMHEALHNHYTQKSLSLSPGK

SEQ ID NO: 15 - protein, 214 aa, synthetic construct
  REGION 1..214: note = Antibody A light chain full-length amino acid sequence (no signalsequence)
SSELTQDPAVSVALGQTVRITCQGDSLRSYYASWYQQKPGQAPVLVIYGKNNRPSGIPDRFSGSSSGNTASLTITGAQAEDEADYYCQSYYSSSHYVVFGGGTKLTVLGQPKAAPSVTLFPPSSEELQANKATLVCLISDFYPGAVTVAWKADSSPVKAGVETTTPSKQSNNKYAASSYLSLTPEQWKSHRSYSCQVTHEGSTVEKTVAPTECS

SEQ ID NO: 16 - DNA, 1347 bp, synthetic construct
  misc_feature 1..1347: note = Antibody A heavy chain full-length gene sequence (no signalsequence)
  source 1..1347: mol_type = other DNA
gaagtgcagctgctggaatccgggggagggctggtgcagcccggcggctctctgagactgtcctgtgctgcctccggcttcaccttttccagctacgctatgtcttgggtgcggcaggctcctggcaagggactggagtgggtgtctgctatcagcggctctggcggctccacatactatgccgacagcgtgaagggcaggttcaccatctctcgggataactccaagaatacactgtatctgcagatgaactctctgagggctgaggacaccgccgtgtactattgcgctcggtactggatctggtggcactatggatttgacgtgtggggacagggcaccctggtgacagtgtcttccgcctccacaaagggaccatccgtgttcccactggccccaagctctaagtccaccagcggcggcacagccgctctgggctgtctggtgaaggactacttccctgagccagtgaccgtgagctggaactctggcgctctgacctccggcgtgcatacatttccagccgtgctgcagtccagcggcctgtacagcctgtcttccgtggtgaccgtgcccagctcttccctgggcacccagacatatatctgcaacgtgaatcacaagcctagcaatacaaaggtggacaagagagtggagccaaagtcttgtgataagacccatacatgccctccatgtcctgccccacccgccgctgccccttccgtgttcctgtttcctccaaagccaaaggacaccctgatgatctctcgcacccctgaggtgacatgcgtggtggtggacgtgagccacgaggatcctgaggtgcagtttaactggtacgtggatggcgtggaggtgcataatgctaagacaaagccaagagaggagcagttcaactctacctttcgcgtggtgtccgtgctgacagtggtgcaccaggattggctgaacggcaaggagtataagtgcaaggtgtctaataagggcctgcccgcccctatcgagaagaccatctccaagacaaagggccagcctagagagccacaggtgtacaccctgcccccttctcgcgaggagatgaccaagaaccaggtgtccctgacatgtctggtgaagggcttctatccctccgacatcgctgtggagtgggagagcaatggccagcctgagaacaattacaagaccacaccacccatgctggactccgatggcagcttctttctgtatagcaagctgaccgtggataagtctaggtggcagcagggcaacgtgttctcctgttccgtgatgcacgaagccctgcacaaccattatactcagaagagcctgtccctgtcccctggcaaa

SEQ ID NO: 17 - DNA, 642 bp, synthetic construct
  misc_feature 1..642: note = Antibody A light chain full-length gene sequence (no signalsequence)
  source 1..642: mol_type = other DNA
tctagtgaactgacccaggatcccgccgtctctgtggccctgggccagacagtgagaatcacctgccagggcgactctctgcgctcctactatgcctcttggtaccagcagaagccaggccaggctcccgtgctggtcatctacggcaagaacaataggccttccggcatcccagatcggtttagcggctccagctctggcaacacagccagcctgacaattacaggagctcaggctgaggatgaggctgattactattgccagtcttactattccagctctcactacgtggtgttcgggggagggacaaagctgaccgtgctgggacagccaaaggctgctccttctgtgaccctgtttcccccttccagcgaggagctgcaggccaataaggccaccctggtgtgcctgatcagcgacttctatccaggagctgtgacagtggcttggaaggctgattcttccccagtgaaggctggcgtggagaccacaacccccagcaagcagtctaacaataagtacgccgcctcctcttatctgtctctgacaccagagcagtggaagtcccataggtcctacagctgccaggtgacccacgaaggtagcacagtcgaaaaaaccgtcgcccccacagagtgttct

SEQ ID NO: 18 - protein, 8 aa, synthetic construct
  REGION 1..8: note = Antibody A heavy chain CDR1
GFTFSSYA

SEQ ID NO: 19 - protein, 8 aa, synthetic construct
  REGION 1..8: note = Antibody A heavy chain CDR2
ISGSGGST

SEQ ID NO: 20 - protein, 13 aa, synthetic construct
  REGION 1..13: note = Antibody A heavy chain CDR3
ARYWIWWHYGFDV

SEQ ID NO: 21 - protein, 6 aa, synthetic construct
  REGION 1..6: note = Antibody A light chain CDR1
SLRSYY

SEQ ID NO: 22 - protein, 11 aa, synthetic construct
  REGION 1..11: note = Antibody A light chain CDR3
QSYYSSSHYVV

SEQ ID NO: 23 - DNA, 24 bp, synthetic construct
  misc_feature 1..24: note = Antibody A heavy chain CDR1
  source 1..24: mol_type = other DNA
ggcttcaccttttccagctacgct

SEQ ID NO: 24 - DNA, 24 bp, synthetic construct
  misc_feature 1..24: note = Antibody A heavy chain CDR2
  source 1..24: mol_type = other DNA
atcagcggctctggcggctccaca

SEQ ID NO: 25 - DNA, 39 bp, synthetic construct
  misc_feature 1..39: note = Antibody A heavy chain CDR3
  source 1..39: mol_type = other DNA
gctcggtactggatctggtggcactatggatttgacgtg

SEQ ID NO: 26 - DNA, 18 bp, synthetic construct
  misc_feature 1..18: note = Antibody A light chain CDR1
  source 1..18: mol_type = other DNA
tctctgcgctcctactat

SEQ ID NO: 27 - DNA, 33 bp, synthetic construct
  misc_feature 1..33: note = Antibody A light chain CDR3
  source 1..33: mol_type = other DNA
cagtcttactattccagctctcactacgtggtg

SEQ ID NO: 28 - protein, 8 aa, synthetic construct
  REGION 1..8: note = Antifolate receptor alpha antibody heavy chain CDR1
GFTFSGYG

SEQ ID NO: 29 - protein, 8 aa, synthetic construct
  REGION 1..8: note = Antifolate receptor alpha antibody heavy chain CDR2
ISSGGSYT

SEQ ID NO: 30 - protein, 12 aa, synthetic construct
  REGION 1..12: note = Antifolate receptor alpha antibody heavy chain CDR3
ARHGDDPAWFAY

SEQ ID NO: 31 - protein, 7 aa, synthetic construct
  REGION 1..7: note = Antifolate receptor alpha antibody light chain CDR1
SSISSNN

SEQ ID NO: 32 - protein, 11 aa, synthetic construct
  REGION 1..11: note = Antifolate receptor alpha antibody light chain CDR3
QQWSSYPYMYT

SEQ ID NO: 33 - protein, 119 aa, synthetic construct
  REGION 1..119: note = Antifolate receptor alpha antibody heavy chain variable region
EVQLVESGGGVVQPGRSLRLSCSASGFTFSGYGLSWVRQAPGKGLEWVAMISSGGSYTYYADSVKGRFAISRDNAKNTLFLQMDSLRPEDTGVYFCARHGDDPAWFAYWGQGTPVTVSS

SEQ ID NO: 34 - protein, 110 aa, synthetic construct
  REGION 1..110: note = Antifolate receptor alpha antibody light chain variable region
DIQLTQSPSSLSASVGDRVTITCSVSSSISSNNLHWYQQKPGKAPKPWIYGTSNLASGVPSRFSGSGSGTDYTFTISSLQPEDIATYYCQQWSSYPYMYTFGQGTKVEIK

SEQ ID NO: 35 - protein, 449 aa, synthetic construct
  REGION 1..449: note = Antifolate receptor alpha antibody heavy chain full-length aminoacid sequence (no signal sequence)
EVQLVESGGGVVQPGRSLRLSCSASGFTFSGYGLSWVRQAPGKGLEWVAMISSGGSYTYYADSVKGRFAISRDNAKNTLFLQMDSLRPEDTGVYFCARHGDDPAWFAYWGQGTPVTVSSASTKGPSVFPLAPSSKSTSGGTAALGCLVKDYFPEPVTVSWNSGALTSGVHTFPAVLQSSGLYSLSSVVTVPSSSLGTQTYICNVNHKPSNTKVDKKVEPKSCDKTHTCPPCPAPEAAGGSSVFLFPPKPKDTLMISRTPEVTCVVVDVSQEDPEVQFNWYVDGVEVHNAKTKPREEQYNSTYRVVSVLTVLHQDWLNGKEYKCKVSNKALPAPIEKTISKAKGQPREPQVYTLPPSRDELTKNQVSLTCLVKGFYPSDIAVEWESNGQPENNYKTTPPVLDSDGSFFLYSKLTVDKSRWQQGNVFSCSVMHEALHNHYTQKSLSLSPGK

SEQ ID NO: 36 - protein, 217 aa, synthetic construct
  REGION 1..217: note = Antifolate receptor alpha antibody light chain full-length aminoacid sequence (no signal sequence)
DIQLTQSPSSLSASVGDRVTITCSVSSSISSNNLHWYQQKPGKAPKPWIYGTSNLASGVPSRFSGSGSGTDYTFTISSLQPEDIATYYCQQWSSYPYMYTFGQGTKVEIKRTVAAPSVFIFPPSDEQLKSGTASVVCLLNNFYPREAKVQWKVDNALQSGNSQESVTEQDSKDSTYSLSSTLTLSKADYEKHKVYACEVTHQGLSSPVTKSFNRGEC

SEQ ID NO: 37 - protein, 19 aa, synthetic construct
  REGION 1..19: note = Antifolate receptor alpha antibody signal sequence
MGWSCIILFLVATATGVHS

SEQ ID NO: 38 - protein, 8 aa, synthetic construct
  REGION 1..8: note = Anti-mesothelin antibody heavy chain CDR1
GIDLSSYA

SEQ ID NO: 39 - protein, 7 aa, synthetic construct
  REGION 1..7: note = Anti-mesothelin antibody heavy chain CDR2
IDISGNR

SEQ ID NO: 40 - protein, 13 aa, synthetic construct
  REGION 1..13: note = Anti-mesothelin antibody heavy chain CDR3
ARVDSRAWGPFNL

SEQ ID NO: 41 - protein, 6 aa, synthetic construct
  REGION 1..6: note = Anti-mesothelin antibody light chain CDR1
QSIFSY

SEQ ID NO: 42 - protein, 12 aa, synthetic construct
  REGION 1..12: note = Anti-mesothelin antibody light chain CDR3
QQGYTRSDVDNA

SEQ ID NO: 43 - protein, 119 aa, synthetic construct
  REGION 1..119: note = Anti-mesothelin antibody heavy chain variable region
QVQLVESGGGVVQPGRSLRLSCAASGIDLSSYAMSWVRQAPGKGLEWIGVIDISGNRFYADWVKGRFTISRDNSKNTLYLQMSSLRAEDTAVYYCARVDSRAWGPFNLWGQGTLVTVSS

SEQ ID NO: 44 - protein, 330 aa, synthetic construct
  REGION 1..330: note = Anti-mesothelin antibody light chain variable region
GATTACCAGATGACCCAGTCCCCCTCCAGCCTGTCCGCTTCTGTGGGCGACAGAGTGACCATCACCTGTCAGGCCTCCCAGTCCATCTTCTCCTACCTGGCCTGGTATCAGCAGAAGCCCGGCAAGGCCCCCAAGCTGCTGATCTACGACGCCTCTGATCTGGCCTCCGGCGTGCCCTCTAGATTCTCCGGCTCTGGCTCTGGCACCGACTTTACCCTGACCATCAGCTCCCTCCAGCCCGAGGATTTCGCCACCTACTACTGCCAGCAGGGCTACACCAGATCCGACGTGGACAACGCCTTTGGCGGAGGCACCAAGGTGGAAATCAAA

SEQ ID NO: 45 - protein, 449 aa, synthetic construct
  REGION 1..449: note = Anti-mesothelin antibody heavy chain full-length amino acidsequence (no signal sequence)
QVQLVESGGGVVQPGRSLRLSCAASGIDLSSYAMSWVRQAPGKGLEWIGVIDISGNRFYADWVKGRFTISRDNSKNTLYLQMSSLRAEDTAVYYCARVDSRAWGPFNLWGQGTLVTVSSASTKGPSVFPLAPSSKSTSGGTAALGCLVKDYFPEPVTVSWNSGALTSGVHTFPAVLQSSGLYSLSSVVTVPSSSLGTQTYICNVNHKPSNTKVDKKVEPKSCDKTHTCPPCPAPEAAGGSSVFLFPPKPKDTLMISRTPEVTCVVVDVSQEDPEVQFNWYVDGVEVHNAKTKPREEQYNSTYRVVSVLTVLHQDWLNGKEYKCKVSNKALPAPIEKTISKAKGQPREPQVYTLPPSRDELTKNQVSLTCLVKGFYPSDIAVEWESNGQPENNYKTTPPVLDSDGSFFLYSKLTVDKSRWQQGNVFSCSVMHEALHNHYTQKSLSLSPGK

SEQ ID NO: 46 - protein, 217 aa, synthetic construct
  REGION 1..217: note = Anti-mesothelin antibody light chain full-length amino acidsequence (no signal sequence)
DYQMTQSPSSLSASVGDRVTITCQASQSIFSYLAWYQQKPGKAPKLLIYDASDLASGVPSRFSGSGSGTDFTLTISSLQPEDFATYYCQQGYTRSDVDNAFGGGTKVEIKRTVAAPSVFIFPPSDEQLKSGTASVVCLLNNFYPREAKVQWKVDNALQSGNSQESVTEQDSKDSTYSLSSTLTLSKADYEKHKVYACEVTHQGLSSPVTKSFNRGEC

SEQ ID NO: 47 - protein, 19 aa, synthetic construct
  REGION 1..19: note = Anti-mesothelin antibody signal sequence
MGWSCIILFLVATATGVHS

SEQ ID NO: 48 - protein, 454 aa, synthetic construct
  REGION 1..454: note = Full length amino acid sequence of anti-FLT3 antibody heavy chain
EEVQLVESGGGLVRPGGSLRLSCAASGFTFSGYSINWVRQAPGKGLEWVSSISSSSNYIYYADSVKGRFTISRDNAKNSLYLQMNSLRAEDTAVYYCAREGFIAGTTFDAFDIWGQGTMVTVSSASTKGPSVFPLAPSSKSTSGGTAALGCLVKDYFPEPVTVSWNSGALTSGVHTFPAVLQSSGLYSLSSVVTVPSSSLGTQTYICNVNHKPSNTKVDKKVEPKSCDKTHTCPPCPAPELLGGPSVFLFPPKPKDTLMISRTPEVTCVVVDVSHEDPEVKFNWYVDGVEVHNAKTKPREEQYNSTYRVVSVLTVLHQDWLNGKEYKCKVSNKALPAPIEKTISKAKGQPREPQVYTLPPSREEMTKNQVSLTCLVKGFYPSDIAVEWESNGQPENNYKTTPPVLDSDGSFFLYSKLTVDKSRWQQGNVFSCSVMHEALHNHYTQKSLSLSPGK

SEQ ID NO: 49 - protein, 215 aa, synthetic construct
  REGION 1..215: note = Full length amino acid sequence of anti-FLT3 antibody light chain
EDIQMTQSPSSLSASVGDRVTITCRASQGIRNDLGWYQQKPGKAPKRLIYAASSLQSGVPSRFSGSGSGTEFTLTISSLQPEDFATYYCLQHNGFPYTFGQGTKLEIKRTVAAPSVFIFPPSDEQLKSGTASVVCLLNNFYPREAKVQWKVDNALQSGNSQESVTEQDSKDSTYSLSSTLTLSKADYEKHKVYACEVTHQGLSSPVTKSFNRGEC

SEQ ID NO: 50 - protein, 448 aa, synthetic construct
  REGION 1..448: note = Full length amino acid sequence of anti-DLL3 antibody heavy chain
EQVQLVQSGAEVKKPGASVKVSCKASGYTFTNYGMNWVRQAPGQGLEWMGWINTYTGEPTYADDFKGRVTMTTDTSTSTAYMELRSLRSDDTAVYYCARIGDSSPSDYWGQGTLVTVSSASTKGPSVFPLAPSSKSTSGGTAALGCLVKDYFPEPVTVSWNSGALTSGVHTFPAVLQSSGLYSLSSVVTVPSSSLGTQTYICNVNHKPSNTKVDKKVEPKSCDKTHTCPPCPAPELLGGPSVFLFPPKPKDTLMISRTPEVTCVVVDVSHEDPEVKFNWYVDGVEVHNAKTKPREEQYNSTYRVVSVLTVLHQDWLNGKEYKCKVSNKALPAPIEKTISKAKGQPREPQVYTLPPSRDELTKNQVSLTCLVKGFYPSDIAVEWESNGQPENNYKTTPPVLDSDGSFFLYSKLTVDKSRWQQGNVFSCSVMHEALHNHYTQKSLSLSPG

SEQ ID NO: 51 - protein, 215 aa, synthetic construct
  REGION 1..215: note = Full length amino acid sequence of anti-DLL3 antibody light chain
EEIVMTQSPATLSVSPGERATLSCKASQSVSNDVVWYQQKPGQAPRLLIYYASNRYTGIPARFSGSGSGTEFTLTISSLQSEDFAVYYCQQDYTSPWTFGQGTKLEIKRTVAAPSVFIFPPSDEQLKSGTASVVCLLNNFYPREAKVQWKVDNALQSGNSQESVTEQDSKDSTYSLSSTLTLSKADYEKHKVYACEVTHQGLSSPVTKSFNRGEC

SEQ ID NO: 52 - protein, 446 aa, synthetic construct
  REGION 1..446: note = Anti-CLDN6 antibody heavy chain full length amino acid sequence
EEVQLQQSGPELVKPGASMKISCKASGYSFTGYTMNWVKQSHGKNLEWIGLINPYNGGTIYNQKFKGKATLTVDKSSSTAYMELLSLTSEDSAVYYCARDYGFVLDYWGQGTTLTVSSASTKGPSVFPLAPSSKSTSGGTAALGCLVKDYFPEPVTVSWNSGALTSGVHTFPAVLQSSGLYSLSSVVTVPSSSLGTQTYICNVNHKPSNTKVDKRVEPKSCDKTHTCPPCPAPPAAAPSVFLFPPKPKDTLMISRTPEVTCVVVDVSHEDPEVQFNWYVDGVEVHNAKTKPREEQFNSTFRVVSVLTVVHQDWLNGKEYKCKVSNKGLPAPIEKTISKTKGQPREPQVYTLPPSREEMTKNQVSLTCLVKGFYPSDIAVEWESNGQPENNYKTTPPMLDSDGSFFLYSKLTVDKSRWQQGNVFSCSVMHEALHNHYTQKSLSLSPG

SEQ ID NO: 53 - protein, 215 aa, synthetic construct
  REGION 1..215: note = Anti-CLDN6 antibody light chain full length amino acid sequence
EQIVLTQSPAIMSASPGEKVTITCSASSSVSYLHWFQQKPGTSPKLWVYSTSNLPSGVPARFGGSGSGTSYSLTISRMEAEDAATYYCQQRSIYPPWTFGGGTKLEIKRTVAAPSVFIFPPSDEQLKSGTASVVCLLNNFYPREAKVQWKVDNALQSGNSQESVTEQDSKDSTYSLSSTLTLSKADYEKHKVYACEVTHQGLSSPVTKSFNRGEC

SEQ ID NO: 54 - protein, 447 aa, synthetic construct
  REGION 1..447: note = Anti-Nectin4 antibody heavy chain full length amino acid sequence
EEVQLVESGGGLVQPGGSLRLSCAASGFTFSSYNMNWVRQAPGKGLEWVSYISSSSSTIYYADSVKGRFTISRDNAKNSLSLQMNSLRDEDTAVYYCARAYYYGMDVWGQGTTVTVSSASTKGPSVFPLAPSSKSTSGGTAALGCLVKDYFPEPVTVSWNSGALTSGVHTFPAVLQSSGLYSLSSVVTVPSSSLGTQTYICNVNHKPSNTKVDKRVEPKSCDKTHTCPPCPAPPAAAPSVFLFPPKPKDTLMISRTPEVTCVVVDVSHEDPEVQFNWYVDGVEVHNAKTKPREEQFNSTFRVVSVLTVVHQDWLNGKEYKCKVSNKGLPAPIEKTISKTKGQPREPQVYTLPPSREEMTKNQVSLTCLVKGFYPSDIAVEWESNGQPENNYKTTPPMLDSDGSFFLYSKLTVDKSRWQQGNVFSCSVMHEALHNHYTQKSLSLSPGK

SEQ ID NO: 55 - protein, 215 aa, synthetic construct
  REGION 1..215: note = Anti-Nectin4 antibody light chain full length amino acid sequence
EDIQMTQSPSSVSASVGDRVTITCRASQGISGWLAWYQQKPGKAPKFLIYAASTLQSGVPSRFSGSGSGTDFTLTISSLQPEDFATYYCQQANSFPPTFGGGTKVEIKRTVAAPSVFIFPPSDEQLKSGTASVVCLLNNFYPREAKVQWKVDNALQSGNSQESVTEQDSKDSTYSLSSTLTLSKADYEKHKVYACEVTHQGLSSPVTKSFNRGEC

SEQ ID NO: 56 - protein, 452 aa, synthetic construct
  REGION 1..452: note = Full length amino acid sequence of anti-TROP2 antibody heavychain
EQVQLQQSGSELKKPGASVKVSCKASGYTFTNYGMNWVKQAPGQGLKWMGWINTYTGEPTYTDDFKGRFAFSLDTSVSTAYLQISSLKADDTAVYFCARGGFGSSYWYFDVWGQGSLVTVSSASTKGPSVFPLAPSSKSTSGGTAALGCLVKDYFPEPVTVSWNSGALTSGVHTFPAVLQSSGLYSLSSVVTVPSSSLGTQTYICNVNHKPSNTKVDKRVEPKSCDKTHTCPPCPAPELLGGPSVFLFPPKPKDTLMISRTPEVTCVVVDVSHEDPEVKFNWYVDGVEVHNAKTKPREEQYNSTYRVVSVLTVLHQDWLNGKEYKCKVSNKALPAPIEKTISKAKGQPREPQVYTLPPSREEMTKNQVSLTCLVKGFYPSDIAVEWESNGQPENNYKTTPPVLDSDGSFFLYSKLTVDKSRWQQGNVFSCSVMHEALHNHYTQKSLSLSPGK

SEQ ID NO: 57 - protein, 215 aa, synthetic construct
  REGION 1..215: note = Full length amino acid sequence of anti-TROP2 antibody lightchain
EDIQLTQSPSSLSASVGDRVSITCKASQDVSIAVAWYQQKPGKAPKLLIYSASYRYTGVPDRFSGSGSGTDFTLTISSLQPEDFAVYYCQQHYITPLTFGAGTKVEIKRTVAAPSVFIFPPSDEQLKSGTASVVCLLNNFYPREAKVQWKVDNALQSGNSQESVTEQDSKDSTYSLSSTLTLSKADYEKHKVYACEVTHQGLSSPVTKSFNRGEC

SEQ ID NO: 58 - protein, 456 aa, synthetic construct
  REGION 1..456: note = Full length amino acid sequence of anti-CA9 antibody heavy chain
EQVQLVESGGGLVQPGGSLRLSCSASGFSLNSYAMIWVRQAPGKGLEYIGFITTGGTTYYADSVKGRFTISRDNSKNTLYLQMNSLRAEDTAVYYCARDRVKSYDDYGDLDAFEPWGQGTLVTVSSASTKGPSVFPLAPSSKSTSGGTAALGCLVKDYFPEPVTVSWNSGALTSGVHTFPAVLQSSGLYSLSSVVTVPSSSLGTQTYICNVNHKPSNTKVDKKVEPKSCDKTHTCPPCPAPELLGGPSVFLFPPKPKDTLMISRTPEVTCVVVDVSHEDPEVKFNWYVDGVEVHNAKTKPREEQYNSTYRVVSVLTVLHQDWLNGKEYKCKVSNKALPAPIEKTISKAKGQPREPQVYTLPPSRDELTKNQVSLTCLVKGFYPSDIAVEWESNGQPENNYKTTPPVLDSDGSFFLYSKLTVDKSRWQQGNVFSCSVMHEALHNHYTQKSLSLSPGK

SEQ ID NO: 59 - protein, 219 aa, synthetic construct
  REGION 1..219: note = Full length amino acid sequence of anti-CA9 antibody light chain
EDIQMTQSPSTLSASVGDRVTITCQASQSISSYLAWYQQKPGKAPKLLIYYASTLASGVPSRFSGSGSGTEFTLTISSLQCDDAATYYCLGVYGYSFDDGIAFGGGTKVEIKRTVAAPSVFIFPPSDEQLKSGTASVVCLLNNFYPREAKVQWKVDNALQSGNSQESVTEQDSKDSTYSLSSTLTLSKADYEKHKVYACEVTHQGLSSPVTKSFNRGEC

SEQ ID NO: 60 - protein, 445 aa, synthetic construct
  REGION 1..445: note = Full length amino acid sequence of anti-CLDN3/4 antibody heavychain
EEVQLEQSGGGLVEPGRSLKLTCAASGFTFSDYNMAWVRQAPTKGLEWVATIIYDGSRTYYRDSVKGRFTISRDNAKSTLYLQMDSLRSADTATYYCTIIGWENWGQGVMVTVSSASTKGPSVFPLAPSSKSTSGGTAALGCLVKDYFPEPVTVSWNSGALTSGVHTFPAVLQSSGLYSLSSVVTVPSSSLGTQTYICNVNHKPSNTKVDKKVEPKSCDKTHTCPPCPAPELLGGPSVFLFPPKPKDTLMISRTPEVTCVVVDVSHEDPEVKFNWYVDGVEVHNAKTKPREEQYNSTYRVVSVLTVLHQDWLNGKEYKCKVSNKALPAPIEKTISKAKGQPREPQVYTLPPSRDELTKNQVSLTCLVKGFYPSDIAVEWESNGQPENNYKTTPPVLDSDGSFFLYSKLTVDKSRWQQGNVFSCSVMHEALHNHYTQKSLSLSPGK

SEQ ID NO: 61 - protein, 221 aa, synthetic construct
  REGION 1..221: note = Full length amino acid sequence of anti-CLDN3/4 antibody lightchain
EDIVLTQSTPTLSATIGQSVSISCRSSQSLLHINGNTYLNWLLQRPGQPPQLLISLVSRLESGVPNRFSGSGSGTDFTLKISGVEAEDLGLYYCGQISHAPPWTFGGGTKLELKRTVAAPSVFIFPPSDEQLKSGTASVVCLLNNFYPREAKVQWKVDNALQSGNSQESVTEQDSKDSTYSLSSTLTLSKADYEKHKVYACEVTHQGLSSPVTKSFNRGEC